European Patent Application EP 4 768 590 A1, published July 1, 2026. Title: Microorganisms introduced with a protein encoded by a foreign ftsN gene and a method for producing L-amino acids using the same. Applicant: CJ CheilJedang Corporation. Application KR. The sequence listing filed with the application follows.

SEQUENCE LISTING (11 sequences)

SEQ ID NO: 1 - DNA, 39 bp, synthetic construct
  source 1..39: mol_type = other DNA
tcgagctcggtaccctaataattctgcttcccgacgatg

SEQ ID NO: 2 - DNA, 40 bp, synthetic construct
  source 1..40: mol_type = other DNA
ctcttccggttcccgggacggtcgatgtcgaggcgttaca

SEQ ID NO: 3 - DNA, 40 bp, synthetic construct
  source 1..40: mol_type = other DNA
ctcgacatcgaccgtcccgggaaccggaagagcccgattg

SEQ ID NO: 4 - DNA, 40 bp, synthetic construct
  source 1..40: mol_type = other DNA
ctctagaggatccccgaaaaggaagaagtctgagaagaag

SEQ ID NO: 5 - DNA, 41 bp, synthetic construct
  source 1..41: mol_type = other DNA
cgacatcgaccgtcccagaaacatcccagcgctactaatag

SEQ ID NO: 6 - DNA, 25 bp, synthetic construct
  source 1..25: mol_type = other DNA
gagtgtttcctttcgttgggtacgt

SEQ ID NO: 7 - DNA, 41 bp, synthetic construct
  source 1..41: mol_type = other DNA
cgaaaggaaacactcgtggcacaacgagattatgtacgccg

SEQ ID NO: 8 - DNA, 40 bp, synthetic construct
  source 1..40: mol_type = other DNA
gctcttccggttccctcaacccccggcggcgagccgaatg

SEQ ID NO: 9 - protein, 319 aa, Escherichia coli
MAQRDYVRRSQPAPSRRKKSTSRKKQRNLPAVSPAMVAIAAAVLVTFIGGLYFITHHKKEESETLQSQKVTGNGLPPKPEERWRYIKELESRQPGVRAPTEPSAGGEVKTPEQLTPEQRQLLEQMQADMRQQPTQLVEVPWNEQTPEQRQQTLQRQRQAQQLAEQQRLAQQSRTTEQSWQQQTRTSQAAPVQAQPRQSKPASSQQPYQDLLQTPAHTTAQSKPQQAAPVARAADAPKPTAEKKDERRWMVQCGSFRGAEQAETVRAQLAFEGFDSKITTNNGWNRVVIGPVKGKENADSTLNRLKMAGHTNCIRLAAGG

SEQ ID NO: 10 - DNA, 960 bp, Escherichia coli
  source 1..960: mol_type = genomic DNA
gtggcacaacgagattatgtacgccgcagccaaccggcaccttcgcggcgaaaaaagagcacctcacggaaaaagcaacgaaatctgcctgcggtttctcccgctatggtcgctattgctgccgccgttcttgtgacctttatcggtggtctgtacttcattacgcatcacaagaaagaagagtccgagacgctgcaaagccagaaagtgaccggaaacggactaccaccaaaaccagaagaacgctggcgctacattaaagagctggaaagtcgccagccgggagtgcgtgcgcccacagaaccttctgccggtggtgaagtgaaaacgccggagcaactgacaccagaacaacgtcagcttcttgaacaaatgcaggctgatatgcgccagcagccaacgcagctggttgaagttccgtggaatgaacagacgccggaacagcgtcagcaaacgctacagcgccaacgtcaggcgcagcaattagcggaacagcaacgcctggctcagcagtcgcgtacgactgaacaaagctggcagcagcagacgcgtacgtcgcaagccgcaccggtacaggcgcaaccgcgccagtctaaaccggcttcttctcagcagccgtaccaggatctgctgcaaactcctgcgcacacgactgcgcagtcgaagccgcagcaagctgcgccagttgctcgtgccgctgacgcgccaaaaccgacggcggagaaaaaagacgaacgccgctggatggtgcagtgcggttcgttcagaggcgcggaacaggcagagacggtacgtgctcagctggcgttcgaaggctttgactcgaaaatcaccaccaacaatggctggaatcgtgtggtcattggcccggtgaaaggcaaagagaacgcagacagcaccctcaatcggttgaagatggcgggtcatacaaactgcattcggctcgccgccgggggttga

SEQ ID NO: 11 - DNA, 5802 bp, synthetic construct
  source 1..5802: mol_type = other DNA
gttcgcttgctgtccataaaaccgcccagtctagctatcgccatgtaagcccactgcaagctacctgctttctctttgcgcttgcgttttcccttgtccagatagcccagtagctgacattcatccggggtcagcaccgtttctgcggactggctttctacgtgttccgcttcctttagcagcccttgcgccctgagtgcttgcggcagcgtgaagctagcttttatcgccattcgccattcaggctgcgcaactgttgggaagggcgatcggtgcgggcctcttcgctattacgccagctggcgaaagggggatgtgctgcaaggcgattaagttgggtaacgccagggttttcccagtcacgacgttgtaaaacgacggccagtgaattcgagctcggtacccggggatcctctagagtcgacctgcaggcatgcaagcttggcgtaatcatggtcatagctgtttcctgtgtgaaattgttatccgctcacaattccacacaacatacgagccggaagcataaagtgtaaagcctggggtgcctaatgagtgagctaactcacattaattgcgttgcgctcactgcccgctttccagtcgggaaacctgtcgtgccagctgcattaatgaatcggccaacgcgcggggagaggcggtttgcgtattgggcgctcttccgcttcctcgctcactgactcgctgcgctcggtcgttcggctgcggcgagcggtatcagctcactcaaaggcggtaatacggttatccacagaatcaggggataacgcaggaaagaacatgtgagcaaaaggccagcaaaaggccaggaaccgtaaaaaggccgcgttgctggcgtttttccataggctccgcccccctgacgagcatcacaaaaatcgacgctcaagtcagaggtggcgaaacccgacaggactataaagataccaggcgtttccccctggaagctccctcgtgcgctctcctgttccgaccctgccgcttaccggatacctgtccgcctttctcccttcgggaagcgtggcgctttctcaatgctcacgctgtaggtatctcagttcggtgtaggtcgttcgctccaagctgggctgtgtgcacgaaccccccgttcagcccgaccgctgcgccttatccggtaactatcgtcttgagtccaacccggtaagacacgacttatcgccactggcagcagccactggtaacaggattagcagagcgaggtatgtaggcggtgctacagagttcttgaagtggtggcctaactacggctacactagaaggacagtatttggtatctgcgctctgctgaagccagttaccttcggaaaaagagttggtagctcttgatccggcaaacaaaccaccgctggtagcggtggtttttttgtttgcaagcagcagattacgcgcagaaaaaaaggatctcaagaagatcctttgatcttttctacggggtctgacgctcagtggaacgaaaactcacgttaagggattttggtcatgagattatcaaaaaggatcttcacctagatccttttggggtgggcgaagaactccagcatgagatccccgcgctggaggatcatccagccctgatagaaacagaagccactggagcacctcaaaaacaccatcatacactaaatcagtaagttggcagcatcacccgacgcactttgcgccgaataaatacctgtgacggaagatcacttcgcagaataaataaatcctggtgtccctgttgataccgggaagccctgggccaacttttggcgaaaatgagacgttgatcggcacgtaagaggttccaactttcaccataatgaaataagatcactaccgggcgtattttttgagttatcgagattttcaggagctgatagaaacagaagccactggagcacctcaaaaacaccatcatacactaaatcagtaagttggcagcatcacccgacgcactttgcgccgaataaatacctgtgacggaagatcacttcgcagaataaataaatcctggtgtccctgttgataccgggaagccctgggccaacttttggcgaaaatgagacgttgatcggcacgtaagaggttccaactttcaccataatgaaataagatcactaccgggcgtattttttgagttatcgagattttcaggagctctttggcatcgtctctcgcctgtcccctcagttcagtaatttcctgcatttgcctgtttccagtcggtagatattccacaaaacagcagggaagcagcgcttttccgctgcataaccctgcttcggggtcattatagcgattttttcggtatatccatcctttttcgcacgatatacaggattttgccaaagggttcgtgtagactttccttggtgtatccaacggcgtcagccgggcaggataggtgaagtaggcccacccgcgagcgggtgttccttcttcactgtcccttattcgcacctggcggtgctcaacgggaatcctgctctgcgaggctggccggctaccgccggcgtaacagatgagggcaagcggatggctgatgaaaccaagccaaccaggaagggcagcccacctatcaaggtgtactgccttccagacgaacgaagagcgattgaggaaaaggcggcggcggccggcatgagcctgtcggcctacctgctggccgtcggccagggctacaaaatcacgggcgtcgtggactatgagcacgtccgcgagggcgtcccggaaaacgattccgaagcccaacctttcatagaaggcggcggtggaatcgaaatctcgtgatggcaggttgggcgtcgcttggtcggtcatttcgaaaaaggttaggaatacggttagccatttgcctgcttttatatagttcatatgggattcacctttatgttgataagaaataaaagaaaatgccaataggatatcggcattttcttttgcgtttttatttgttaactgttaattgtccttgttcaaggatgctgtctttgacaacagatgttttcttgcctttgatgttcagcaggaagctcggcgcaaacgttgattgtttgtctgcgtagaatcctctgtttgtcatatagcttgtaatcacgacattgtttcctttcgcttgaggtacagcgaagtgtgagtaagtaaaggttacatcgttaggcggatcaagatccatttttaacacaaggccagttttgttcagcggcttgtatgggccagttaaagaattagaaacataaccaagcatgtaaatatcgttagacgtaatgccgtcaatcgtcatttttgatccgcgggagtcagtgaacaggtaccatttgccgttcattttaaagacgttcgcgcgttcaatttcatctgttactgtgttagatgcaatcagcggtttcatcacttttttcagtgtgtaatcatcgtttagctcaatcataccgagagcgccgtttgctaactcagccgtgcgttttttatcgctttgcagaagtttttgactttcttgacggaagaatgatgtgcttttgccatagtatgctttgttaaataaagattcttcgccttggtagccatcttcagttccagtgtttgcttcaaatactaagtatttgtggcctttatcttctacgtagtgaggatctctcagcgtatggttgtcgcctgagctgtagttgccttcatcgatgaactgctgtacattttgatacgtttttccgtcaccgtcaaagattgatttataatcctctacaccgttgatgttcaaagagctgtctgatgctgatacgttaacttgtgcagttgtcagtgtttgtttgccgtaatgtttaccggagaaatcagtgtagaataaacggatttttccgtcagatgtaaatgtggctgaacctgaccattcttgtgtttggtcttttaggatagaatcatttgcatcgaatttgtcgctgtctttaaagacgcggccagcgtttttccagctgtcaatagaagtttcgccgactttttgatagaacatgtaaatcgatgtgtcatccgcatttttaggatctccggctaatgcaaagacgatgtggtagccgtgatagtttgcgacagtgccgtcagcgttttgtaatggccagctgtcccaaacgtccaggccttttgcagaagagatatttttaattgtggacgaatcaaattcagaaacttgatatttttcatttttttgctgttcagggatttgcagcatatcatggcgtgtaatatgggaaatgccgtatgtttccttatatggcttttggttcgtttctttcgcaaacgcttgagttgcgcctcctgccagcagtgcggtagtaaaggttaatactgttgcttgttttgcaaactttttgatgttcatcgttcatgtctccttttttatgtactgtgttagcggtctgcttcttccagccctcctgtttgaagatggcaagttagttacgcacaataaaaaaagacctaaaatatgtaaggggtgacgccaaagtatacactttgccctttacacattttaggtcttgcctgctttatcagtaacaaacccgcgcgatttacttttcgacctcattctattagactctcgtttggattgcaactggtctattttcctcttttgtttgatagaaaatcataaaaggatttgcagactacgggcctaaagaactaaaaaatctatctgtttcttttcattctctgtattttttatagtttctgttgcatgggcataaagttgcctttttaatcacaattcagaaaatatcataatatctcatttcactaaataatagtgaacggcaggtatatgtgatgggttaaaaaggatcaccccagagtcccgctcagaagaactcgtcaagaaggcgatagaaggcgatgcgctgcgaatcgggagcggcgataccgtaaagcacgaggaagcggtcagcccattcgccgccaagctcttcagcaatatcacgggtagccaacgctatgtcctgatagcggtccgccacacccagccggccacagtcgatgaatccagaaaagcggccattttccaccatgatattcggcaagcaggcatcgccatgggtcacgacgagatcctcgccgtcgggcatccgcgccttgagcctggcgaacagttcggctggcgcgagcccctgatgctcttcgtccagatcatcctgatcgacaagaccggcttccatccgagtacgtgctcgctcgatgcgatgtttcgcttggtggtcgaatgggcaggtagccggatcaagcgtatgcagccgccgcattgcatcagccatgatggatactttctcggcaggagcaaggtgagatgacaggagatcctgccccggcacttcgcccaatagcagccagtcccttcccgcttcagtgacaacgtcgagacagctgcgcaaggaacgcccgtcgtggccagccacgatagccgcgctgcctcgtcttggagttcattcagggcaccggacaggtcggtcttgacaaaaagaaccgggcgcccctgcgctgacagccggaacacggcggcatcagagcagccgattgtctgttgtgcccagtcatagccgaatagcctctccacccaagcggccggagaacctgcgtgcaatccatcttgttcaatcatgcgaaacgatcctcatcctgtctcttgatcagatcttgatcccctgcgccatcagatccttggcggcaagaaagccatccagtttactttgcagggcttcccaaccttaccagagggcgccccagctggcaattccg